European Patent Application EP 4 455 274 A1, published October 30, 2024. Title: ESTABLISHMENT OF ERYTHROID PRECURSOR CELL LINE CAPABLE OF CONDITIONAL MATURATION USING GENE OVEREXPRESSION. Applicant: IUCF-HYU (INDUSTRY-UNIVERSITY COOPERATION FOUNDATION HANYANG UNIVERSITY). Application IB WO2022KR18737, filed November 24, 2022. The sequence listing filed with the application follows.

SEQUENCE LISTING (12 sequences)

SEQ ID NO: 1 - DNA, 19 bp, unidentified
  source 1..19: mol_type = genomic DNA
gaaggtgaaggtcggagtc

SEQ ID NO: 2 - DNA, 20 bp, unidentified
  source 1..20: mol_type = genomic DNA
gacaagcttcccgttctcag

SEQ ID NO: 3 - DNA, 20 bp, unidentified
  source 1..20: mol_type = genomic DNA
gcgacccagaaagttaccac

SEQ ID NO: 4 - DNA, 22 bp, unidentified
  source 1..22: mol_type = genomic DNA
gcaacaagacatacatcgccgg

SEQ ID NO: 5 - DNA, 22 bp, unidentified
  source 1..22: mol_type = genomic DNA
gcaaccagagacaactgatctc

SEQ ID NO: 6 - DNA, 21 bp, unidentified
  source 1..21: mol_type = genomic DNA
tggggcacacaattcctagtg

SEQ ID NO: 7 - DNA, 21 bp, unidentified
  source 1..21: mol_type = genomic DNA
gtcaaaagccactgtgtcctg

SEQ ID NO: 8 - DNA, 20 bp, unidentified
  source 1..20: mol_type = genomic DNA
gcacaaccgaagcgtagagt

SEQ ID NO: 9 - DNA, 21 bp, unidentified
  source 1..21: mol_type = genomic DNA
gagctggtggttgactttctc

SEQ ID NO: 10 - DNA, 21 bp, unidentified
  source 1..21: mol_type = genomic DNA
tccatctccgattcagtccct

SEQ ID NO: 11 - DNA, 20 bp, unidentified
  source 1..20: mol_type = genomic DNA
ccagggcttttcaaaaatga

SEQ ID NO: 12 - DNA, 20 bp, unidentified
  source 1..20: mol_type = genomic DNA
ccgatccaatctgttctggt